European Patent Application EP 4 279 514 A1, published November 22, 2023. Title: FUSION ENZYME AND USE THEREOF IN PAPER-BASED BIOSENSOR. Applicant: BIOLOGY INSTITUTE OF SHANDONG ACADEMY OF SCIENCES. The sequence listing filed with the application follows.

SEQUENCE LISTING (16 sequences)

SEQ ID NO: 1 - protein, 567 aa, Aspergillus niger
GSPAHYDFVIVGGGTSGLVVADRLSELNNVTVAVIEAGESALNNFNVSNVMGYSTAFGTEVDWAYQTENQTYAGGLQQTIRAGKALGGTSTINGMSYTRAEDVQIDNWEVLGNEGWNWKNLFQYYKKSEGFQVPTKDQIAHGANYNASYHGLNGPLKVGWPTSMTNSSVFPVLEQTFEKLGVQYNPDSEGGKMVGFTVHPDTLDREMNVREDAARAYYWPYEARSNLKIISNTRANKVIWADTTQGEAVAVGIEVTNAYGTQTIYADKEVILSAGALRSPALLELSGIGNPDVLNKHNIPVKVNITTVGENLQDQTNNALSWEGVDTLTGLATFSVLPSVNQLYGDNVTALASYVKSQLASYAKTVADASNGAVKEANLIEAFERQYDLIFNSQVPYAEVVFAPSGQSFAVEYWPLLPFSRGSVHIQSANASDYPAINPNYFMFRQDADAQITVAQYIRKALGTTPLNSLVGEEVSPSLEVLPANASSSTWTKWVQENYRTNYHPVGTNSMLPREKGGVVSPELRVYGTKNLRVVDASVLPFQLCGHLTSTLYAVAERASDLIKESY

SEQ ID NO: 2 - DNA, 1701 bp, Aspergillus niger
ggttctccagctcattacgattttgttattgttggaggtggtactagtggtttggttgttgctaatagattgtctgaattgaataacgttaccgttgctgttattgaggctggtgagtctgctttgaataattttaatgtttccaacgtcatgggttactctactgcttttggtactgaagtcgattgggcttatcagactgaaaatcaaacttatgctggaggtcttcaacaaactattagagccggtaaggctttgggtggtacttctactattaacggaatgtcttatactagagctgaggatgttcaaattgataactgggaagttttgggtaatgaaggttggaactggaagaacttgtttcaatattataagaagtccgagggatttcaagttcctactaaggaccaaattgctcatggtgctaactacaacgctagttaccatggtttgaacggtccattgaaggtcggatggcctacttccatgaccaactcttcagtttttccagttcttgaacaaaccttcgaaaagttgggtgttcaatacaacccagattctgaaggaggtaagatggttggtttcactgttcatccagacactttggacagagaaatgaatgttagagaggatgcagctagagcttactactggccatatgaagctagatccaacttgaagattatttcaaacactagagctaacaaggtcatttgggccgatactacccaaggtgaggctgttgctgttggtattgaagttactaacgcttacggtacacaaaccatctacgctgataaggaagttatcttgtcagctggagcattgagatctcctgctttgttggaattgtctggtattggtaatccagatgttttgaacaagcataacattccagttaaggtcaacattactactgttggtgaaaacttgcaggatcaaactaacaacgctttgtcttgggaaggtgttgataccttgaccggtcttgctactttttctgttttgccatctgttaaccaattgtacggagataatgttactgctttggcttcttatgttaagtcccaattggcttcttacgctaagactgttgctgatgcttctaacggtgctgttaaggaggctaacttgattgaggcttttgaaagacaatatgatttgattttcaactcccaagttccatacgctgaggttgtttttgccccatctggtcaatcttttgcagttgaatattggccattgttgccattttctagaggttctgttcatattcaatctgctaacgcttctgattatccagccattaatccaaattactttatgtttagacaggacgctgatgctcaaattactgttgctcagtacattagaaaggctttgggaactactccacttaattctttggttggtgaagaagtttccccatccttggaagttttgcctgccaacgcttcttcttctacctggaccaagtgggttcaagaaaactacagaactaactaccacccagttggtactaactctatgttgccaagagaaaaaggtggtgttgtttcccctgaattgagagtttacggtactaagaacttgagagttgtcgatgcctctgttttgccttttcaactttgtggtcacttgacttctaccctttacgctgtcgctgaaagagcttccgatttgattaaggaatcttac

SEQ ID NO: 3 - protein, 121 aa, Artificial Sequence
  CBM
PGEPGGPGGPGEPGGPGDGTCAVNYTVVNDWGHGMQGAITVSNTGSSPINNWTLQFSFSGVNISNGWNGEWSQSGSQITVRAPAWNSTLQPGQSVELGFVADKTGNVSPPSQFTLNGATCS

SEQ ID NO: 4 - DNA, 363 bp, Artificial Sequence
  CBM
ccgggtgagccgggcggtcctggcggtccgggtgaaccgggcggccccggtgacggcacctgcgcggtgaactacaccgtggtcaatgactggggtcacggtatgcagggggcgatcaccgtctccaacaccggatcctcgcccatcaacaactggaccctgcagttcagcttctcgggtgtgaacatctccaacggctggaacggcgagtggagccagagcggctcgcagatcaccgtccgcgctcctgcctggaactccacgctccagccgggccagagcgtggaactgggcttcgttgctgacaagaccggcaacgtctccccgccctcccagttcaccctcaacggagccacctgctcc

SEQ ID NO: 5 - protein, 38 aa, Artificial Sequence
  Natural linker
LGGDSSGGGPGEPGGPGGPGEPGGPGGPGEPGGPGDGT

SEQ ID NO: 6 - DNA, 114 bp, Artificial Sequence
  Natural linker
ctcggcggcgactcctccggcggcggtccgggtgagccgggcggtcctggcggtccgggtgagccgggcggtcctggcggtccgggtgaaccgggcggccccggtgacggcacc

SEQ ID NO: 7 - protein, 15 aa, Artificial Sequence
  (EAAAK)3 linker
EAAAKEAAAKEAAAK

SEQ ID NO: 8 - DNA, 45 bp, Artificial Sequence
  (EAAAK)3 linker
gaagctgccgcaaaagaagctgccgcaaaagaagctgccgcaaaa

SEQ ID NO: 9 - protein, 10 aa, Artificial Sequence
  (GGGGS)2 linker
GGGGSGGGGS

SEQ ID NO: 10 - DNA, 30 bp, Artificial Sequence
  (GGGGS)2 linker
ggtggaggtggatctggaggtggtggatct

SEQ ID NO: 11 - protein, 732 aa, Artificial Sequence
  GDH-NL-CBM2
GSPAHYDFVIVGGGTSGLVVADRLSELNNVTVAVIEAGESALNNFNVSNVMGYSTAFGTEVDWAYQTENQTYAGGLQQTIRAGKALGGTSTINGMSYTRAEDVQIDNWEVLGNEGWNWKNLFQYYKKSEGFQVPTKDQIAHGANYNASYHGLNGPLKVGWPTSMTNSSVFPVLEQTFEKLGVQYNPDSEGGKMVGFTVHPDTLDREMNVREDAARAYYWPYEARSNLKIISNTRANKVIWADTTQGEAVAVGIEVTNAYGTQTIYADKEVILSAGALRSPALLELSGIGNPDVLNKHNIPVKVNITTVGENLQDQTNNALSWEGVDTLTGLATFSVLPSVNQLYGDNVTALASYVKSQLASYAKTVADASNGAVKEANLIEAFERQYDLIFNSQVPYAEVVFAPSGQSFAVEYWPLLPFSRGSVHIQSANASDYPAINPNYFMFRQDADAQITVAQYIRKALGTTPLNSLVGEEVSPSLEVLPANASSSTWTKWVQENYRTNYHPVGTNSMLPREKGGVVSPELRVYGTKNLRVVDASVLPFQLCGHLTSTLYAVAERASDLIKESYLGGDSSGGGPGEPGGPGGPGEPGGPGGPGEPGGPGDGTPGEPGGPGGPGEPGGPGDGTCAVNYTVVNDWGHGMQGAITVSNTGSSPINNWTLQFSFSGVNISNGWNGEWSQSGSQITVRAPAWNSTLQPGQSVELGFVADKTGNVSPPSQFTLNGATCSHHHHHH

SEQ ID NO: 12 - DNA, 2199 bp, Artificial Sequence
  GDH-NL-CBM2
ggttctccagctcattacgattttgttattgttggaggtggtactagtggtttggttgttgctaatagattgtctgaattgaataacgttaccgttgctgttattgaggctggtgagtctgctttgaataattttaatgtttccaacgtcatgggttactctactgcttttggtactgaagtcgattgggcttatcagactgaaaatcaaacttatgctggaggtcttcaacaaactattagagccggtaaggctttgggtggtacttctactattaacggaatgtcttatactagagctgaggatgttcaaattgataactgggaagttttgggtaatgaaggttggaactggaagaacttgtttcaatattataagaagtccgagggatttcaagttcctactaaggaccaaattgctcatggtgctaactacaacgctagttaccatggtttgaacggtccattgaaggtcggatggcctacttccatgaccaactcttcagtttttccagttcttgaacaaaccttcgaaaagttgggtgttcaatacaacccagattctgaaggaggtaagatggttggtttcactgttcatccagacactttggacagagaaatgaatgttagagaggatgcagctagagcttactactggccatatgaagctagatccaacttgaagattatttcaaacactagagctaacaaggtcatttgggccgatactacccaaggtgaggctgttgctgttggtattgaagttactaacgcttacggtacacaaaccatctacgctgataaggaagttatcttgtcagctggagcattgagatctcctgctttgttggaattgtctggtattggtaatccagatgttttgaacaagcataacattccagttaaggtcaacattactactgttggtgaaaacttgcaggatcaaactaacaacgctttgtcttgggaaggtgttgataccttgaccggtcttgctactttttctgttttgccatctgttaaccaattgtacggagataatgttactgctttggcttcttatgttaagtcccaattggcttcttacgctaagactgttgctgatgcttctaacggtgctgttaaggaggctaacttgattgaggcttttgaaagacaatatgatttgattttcaactcccaagttccatacgctgaggttgtttttgccccatctggtcaatcttttgcagttgaatattggccattgttgccattttctagaggttctgttcatattcaatctgctaacgcttctgattatccagccattaatccaaattactttatgtttagacaggacgctgatgctcaaattactgttgctcagtacattagaaaggctttgggaactactccacttaattctttggttggtgaagaagtttccccatccttggaagttttgcctgccaacgcttcttcttctacctggaccaagtgggttcaagaaaactacagaactaactaccacccagttggtactaactctatgttgccaagagaaaaaggtggtgttgtttcccctgaattgagagtttacggtactaagaacttgagagttgtcgatgcctctgttttgccttttcaactttgtggtcacttgacttctaccctttacgctgtcgctgaaagagcttccgatttgattaaggaatcttacctcggcggcgactcctccggcggcggtccgggtgagccgggcggtcctggcggtccgggtgagccgggcggtcctggcggtccgggtgaaccgggcggccccggtgacggcaccccgggtgagccgggcggtcctggcggtccgggtgaaccgggcggccccggtgacggcacctgcgcggtgaactacaccgtggtcaatgactggggtcacggtatgcagggggcgatcaccgtctccaacaccggatcctcgcccatcaacaactggaccctgcagttcagcttctcgggtgtgaacatctccaacggctggaacggcgagtggagccagagcggctcgcagatcaccgtccgcgctcctgcctggaactccacgctccagccgggccagagcgtggaactgggcttcgttgctgacaagaccggcaacgtctccccgccctcccagttcaccctcaacggagccacctgctcccaccaccaccaccaccactaa

SEQ ID NO: 13 - protein, 709 aa, Artificial Sequence
  GDH-(EAAAK)3-CBM2
GSPAHYDFVIVGGGTSGLVVADRLSELNNVTVAVIEAGESALNNFNVSNVMGYSTAFGTEVDWAYQTENQTYAGGLQQTIRAGKALGGTSTINGMSYTRAEDVQIDNWEVLGNEGWNWKNLFQYYKKSEGFQVPTKDQIAHGANYNASYHGLNGPLKVGWPTSMTNSSVFPVLEQTFEKLGVQYNPDSEGGKMVGFTVHPDTLDREMNVREDAARAYYWPYEARSNLKIISNTRANKVIWADTTQGEAVAVGIEVTNAYGTQTIYADKEVILSAGALRSPALLELSGIGNPDVLNKHNIPVKVNITTVGENLQDQTNNALSWEGVDTLTGLATFSVLPSVNQLYGDNVTALASYVKSQLASYAKTVADASNGAVKEANLIEAFERQYDLIFNSQVPYAEVVFAPSGQSFAVEYWPLLPFSRGSVHIQSANASDYPAINPNYFMFRQDADAQITVAQYIRKALGTTPLNSLVGEEVSPSLEVLPANASSSTWTKWVQENYRTNYHPVGTNSMLPREKGGVVSPELRVYGTKNLRVVDASVLPFQLCGHLTSTLYAVAERASDLIKESYEAAAKEAAAKEAAAKPGEPGGPGGPGEPGGPGDGTCAVNYTVVNDWGHGMQGAITVSNTGSSPINNWTLQFSFSGVNISNGWNGEWSQSGSQITVRAPAWNSTLQPGQSVELGFVADKTGNVSPPSQFTLNGATCSHHHHHH

SEQ ID NO: 14 - DNA, 2130 bp, Artificial Sequence
  GDH-(EAAAK)3-CBM2
ggttctccagctcattacgattttgttattgttggaggtggtactagtggtttggttgttgctaatagattgtctgaattgaataacgttaccgttgctgttattgaggctggtgagtctgctttgaataattttaatgtttccaacgtcatgggttactctactgcttttggtactgaagtcgattgggcttatcagactgaaaatcaaacttatgctggaggtcttcaacaaactattagagccggtaaggctttgggtggtacttctactattaacggaatgtcttatactagagctgaggatgttcaaattgataactgggaagttttgggtaatgaaggttggaactggaagaacttgtttcaatattataagaagtccgagggatttcaagttcctactaaggaccaaattgctcatggtgctaactacaacgctagttaccatggtttgaacggtccattgaaggtcggatggcctacttccatgaccaactcttcagtttttccagttcttgaacaaaccttcgaaaagttgggtgttcaatacaacccagattctgaaggaggtaagatggttggtttcactgttcatccagacactttggacagagaaatgaatgttagagaggatgcagctagagcttactactggccatatgaagctagatccaacttgaagattatttcaaacactagagctaacaaggtcatttgggccgatactacccaaggtgaggctgttgctgttggtattgaagttactaacgcttacggtacacaaaccatctacgctgataaggaagttatcttgtcagctggagcattgagatctcctgctttgttggaattgtctggtattggtaatccagatgttttgaacaagcataacattccagttaaggtcaacattactactgttggtgaaaacttgcaggatcaaactaacaacgctttgtcttgggaaggtgttgataccttgaccggtcttgctactttttctgttttgccatctgttaaccaattgtacggagataatgttactgctttggcttcttatgttaagtcccaattggcttcttacgctaagactgttgctgatgcttctaacggtgctgttaaggaggctaacttgattgaggcttttgaaagacaatatgatttgattttcaactcccaagttccatacgctgaggttgtttttgccccatctggtcaatcttttgcagttgaatattggccattgttgccattttctagaggttctgttcatattcaatctgctaacgcttctgattatccagccattaatccaaattactttatgtttagacaggacgctgatgctcaaattactgttgctcagtacattagaaaggctttgggaactactccacttaattctttggttggtgaagaagtttccccatccttggaagttttgcctgccaacgcttcttcttctacctggaccaagtgggttcaagaaaactacagaactaactaccacccagttggtactaactctatgttgccaagagaaaaaggtggtgttgtttcccctgaattgagagtttacggtactaagaacttgagagttgtcgatgcctctgttttgccttttcaactttgtggtcacttgacttctaccctttacgctgtcgctgaaagagcttccgatttgattaaggaatcttacgaagctgccgcaaaagaagctgccgcaaaagaagctgccgcaaaaccgggtgagccgggcggtcctggcggtccgggtgaaccgggcggccccggtgacggcacctgcgcggtgaactacaccgtggtcaatgactggggtcacggtatgcagggggcgatcaccgtctccaacaccggatcctcgcccatcaacaactggaccctgcagttcagcttctcgggtgtgaacatctccaacggctggaacggcgagtggagccagagcggctcgcagatcaccgtccgcgctcctgcctggaactccacgctccagccgggccagagcgtggaactgggcttcgttgctgacaagaccggcaacgtctccccgccctcccagttcaccctcaacggagccacctgctcccaccaccaccaccaccactaa

SEQ ID NO: 15 - protein, 704 aa, Artificial Sequence
  GDH-(GGGGS)2-CBM2
GSPAHYDFVIVGGGTSGLVVADRLSELNNVTVAVIEAGESALNNFNVSNVMGYSTAFGTEVDWAYQTENQTYAGGLQQTIRAGKALGGTSTINGMSYTRAEDVQIDNWEVLGNEGWNWKNLFQYYKKSEGFQVPTKDQIAHGANYNASYHGLNGPLKVGWPTSMTNSSVFPVLEQTFEKLGVQYNPDSEGGKMVGFTVHPDTLDREMNVREDAARAYYWPYEARSNLKIISNTRANKVIWADTTQGEAVAVGIEVTNAYGTQTIYADKEVILSAGALRSPALLELSGIGNPDVLNKHNIPVKVNITTVGENLQDQTNNALSWEGVDTLTGLATFSVLPSVNQLYGDNVTALASYVKSQLASYAKTVADASNGAVKEANLIEAFERQYDLIFNSQVPYAEVVFAPSGQSFAVEYWPLLPFSRGSVHIQSANASDYPAINPNYFMFRQDADAQITVAQYIRKALGTTPLNSLVGEEVSPSLEVLPANASSSTWTKWVQENYRTNYHPVGTNSMLPREKGGVVSPELRVYGTKNLRVVDASVLPFQLCGHLTSTLYAVAERASDLIKESYGGGGSGGGGSPGEPGGPGGPGEPGGPGDGTCAVNYTVVNDWGHGMQGAITVSNTGSSPINNWTLQFSFSGVNISNGWNGEWSQSGSQITVRAPAWNSTLQPGQSVELGFVADKTGNVSPPSQFTLNGATCSHHHHHH

SEQ ID NO: 16 - DNA, 2115 bp, Artificial Sequence
  GDH-(GGGGS)2-CBM2
ggttctccagctcattacgattttgttattgttggaggtggtactagtggtttggttgttgctaatagattgtctgaattgaataacgttaccgttgctgttattgaggctggtgagtctgctttgaataattttaatgtttccaacgtcatgggttactctactgcttttggtactgaagtcgattgggcttatcagactgaaaatcaaacttatgctggaggtcttcaacaaactattagagccggtaaggctttgggtggtacttctactattaacggaatgtcttatactagagctgaggatgttcaaattgataactgggaagttttgggtaatgaaggttggaactggaagaacttgtttcaatattataagaagtccgagggatttcaagttcctactaaggaccaaattgctcatggtgctaactacaacgctagttaccatggtttgaacggtccattgaaggtcggatggcctacttccatgaccaactcttcagtttttccagttcttgaacaaaccttcgaaaagttgggtgttcaatacaacccagattctgaaggaggtaagatggttggtttcactgttcatccagacactttggacagagaaatgaatgttagagaggatgcagctagagcttactactggccatatgaagctagatccaacttgaagattatttcaaacactagagctaacaaggtcatttgggccgatactacccaaggtgaggctgttgctgttggtattgaagttactaacgcttacggtacacaaaccatctacgctgataaggaagttatcttgtcagctggagcattgagatctcctgctttgttggaattgtctggtattggtaatccagatgttttgaacaagcataacattccagttaaggtcaacattactactgttggtgaaaacttgcaggatcaaactaacaacgctttgtcttgggaaggtgttgataccttgaccggtcttgctactttttctgttttgccatctgttaaccaattgtacggagataatgttactgctttggcttcttatgttaagtcccaattggcttcttacgctaagactgttgctgatgcttctaacggtgctgttaaggaggctaacttgattgaggcttttgaaagacaatatgatttgattttcaactcccaagttccatacgctgaggttgtttttgccccatctggtcaatcttttgcagttgaatattggccattgttgccattttctagaggttctgttcatattcaatctgctaacgcttctgattatccagccattaatccaaattactttatgtttagacaggacgctgatgctcaaattactgttgctcagtacattagaaaggctttgggaactactccacttaattctttggttggtgaagaagtttccccatccttggaagttttgcctgccaacgcttcttcttctacctggaccaagtgggttcaagaaaactacagaactaactaccacccagttggtactaactctatgttgccaagagaaaaaggtggtgttgtttcccctgaattgagagtttacggtactaagaacttgagagttgtcgatgcctctgttttgccttttcaactttgtggtcacttgacttctaccctttacgctgtcgctgaaagagcttccgatttgattaaggaatcttacggtggaggtggatctggaggtggtggatctccgggtgagccgggcggtcctggcggtccgggtgaaccgggcggccccggtgacggcacctgcgcggtgaactacaccgtggtcaatgactggggtcacggtatgcagggggcgatcaccgtctccaacaccggatcctcgcccatcaacaactggaccctgcagttcagcttctcgggtgtgaacatctccaacggctggaacggcgagtggagccagagcggctcgcagatcaccgtccgcgctcctgcctggaactccacgctccagccgggccagagcgtggaactgggcttcgttgctgacaagaccggcaacgtctccccgccctcccagttcaccctcaacggagccacctgctcccaccaccaccaccaccactaa